European Patent Application EP 4 752 160 A1, published June 3, 2026. Title: 人源化抗CD19单链可变区片段及其用途. Applicant: 星尘股份有限公司. The sequence listing filed with the application follows.

SEQUENCE LISTING (25 sequences)

SEQ ID NO: 1 - protein, 120 aa, synthetic construct
  source 1..120: note = VH4
QVQLQESGPGLVKPSETLSLTCTVSGVSLPDYGVSWIRQPPGKGLEWIGVIWGSETTYYNPSLKSRVTISVDTSKNQVSLKLSSVTAADTAVYYCAKHYYYGGSYAMDYWGQGTTVTVSS

SEQ ID NO: 2 - protein, 120 aa, synthetic construct
  source 1..120: note = VH1
EVQLQESGPGLVKPSETLSVTCTVSGVSLPDYGVSWIRQPPGKGLEWLGVIWGSETTYYNSALKSRLTIIKDNSKSQVFLKMSSLTAADTAVYYCAKHYYYGGSYAMDYWGQGTTVTVSS

SEQ ID NO: 3 - protein, 120 aa, synthetic construct
  source 1..120: note = VH2
QVQLQESGPGLVKPSETLSLTCTVSGVSLPDYGVSWIRQPPGKGLEWLGVIWGSETTYYNSALKSRLTISKDNSKSQVFLKMSSVTAADTAVYYCAKHYYYGGSYAMDYWGQGTTVTVSS

SEQ ID NO: 4 - protein, 120 aa, synthetic construct
  source 1..120: note = VH3
QVQLQESGPGLVKPSETLSLTCTVSGVSLPDYGVSWIRQPPGKGLEWLGVIWGSETTYYNSALKSRVTISVDTSKNQVSLKLSSVTAADTAVYYCAKHYYYGGSYAMDYWGQGTTVTVSS

SEQ ID NO: 5 - protein, 107 aa, synthetic construct
  source 1..107: note = VL3
DIQMTQSPSSLSASVGDRVTITCRASQDISKYLNWYQQKPGKAPKLLIYHTSRLHSGVPSRFSGSGSGTDFTLTISSLQPEDFATYYCQQGNTLPYTFGGGTKLEIK

SEQ ID NO: 6 - protein, 107 aa, synthetic construct
  source 1..107: note = VL1
DIQMTQSPSSLSASVGDRVTISCRASQDISKYLNWYQQKPGKAPKLLIYHTSRLHSGVPSRFSGSGSGTDYTLTISSLQPEDFATYYCQQGNTLPYTFGGGTKLEIK

SEQ ID NO: 7 - protein, 107 aa, synthetic construct
  source 1..107: note = VL2
DIQMTQSPSSLSASVGDRVTITCRASQDISKYLNWYQQKPGKAPKLLIYHTSRLHSGVPSRFSGSGSGTDYTLTISSLQPEDFATYYCQQGNTLPYTFGGGTKLEIK

SEQ ID NO: 8 - protein, 242 aa, synthetic construct
  source 1..242: note = VL3VH4 scFv
DIQMTQSPSSLSASVGDRVTITCRASQDISKYLNWYQQKPGKAPKLLIYHTSRLHSGVPSRFSGSGSGTDFTLTISSLQPEDFATYYCQQGNTLPYTFGGGTKLEIKGGGGSGGGGSGGGGSQVQLQESGPGLVKPSETLSLTCTVSGVSLPDYGVSWIRQPPGKGLEWIGVIWGSETTYYNPSLKSRVTISVDTSKNQVSLKLSSVTAADTAVYYCAKHYYYGGSYAMDYWGQGTTVTVSS

SEQ ID NO: 9 - protein, 242 aa, synthetic construct
  source 1..242: note = VL1VH1 scFv
DIQMTQSPSSLSASVGDRVTISCRASQDISKYLNWYQQKPGKAPKLLIYHTSRLHSGVPSRFSGSGSGTDYTLTISSLQPEDFATYYCQQGNTLPYTFGGGTKLEIKGGGGSGGGGSGGGGSEVQLQESGPGLVKPSETLSVTCTVSGVSLPDYGVSWIRQPPGKGLEWLGVIWGSETTYYNSALKSRLTIIKDNSKSQVFLKMSSLTAADTAVYYCAKHYYYGGSYAMDYWGQGTTVTVSS

SEQ ID NO: 10 - protein, 242 aa, synthetic construct
  source 1..242: note = VL1VH2 scFv
DIQMTQSPSSLSASVGDRVTISCRASQDISKYLNWYQQKPGKAPKLLIYHTSRLHSGVPSRFSGSGSGTDYTLTISSLQPEDFATYYCQQGNTLPYTFGGGTKLEIKGGGGSGGGGSGGGGSQVQLQESGPGLVKPSETLSLTCTVSGVSLPDYGVSWIRQPPGKGLEWLGVIWGSETTYYNSALKSRLTISKDNSKSQVFLKMSSVTAADTAVYYCAKHYYYGGSYAMDYWGQGTTVTVSS

SEQ ID NO: 11 - protein, 5 aa, synthetic construct
  source 1..5: note = Linker
GGGGS

SEQ ID NO: 12 - protein, 4 aa, synthetic construct
  source 1..4: note = Linker
GGGS

SEQ ID NO: 13 - protein, 5 aa, synthetic construct
  source 1..5: note = Linker
SSSSG

SEQ ID NO: 14 - protein, 5 aa, synthetic construct
  source 1..5: note = Linker
GSGSA

SEQ ID NO: 15 - protein, 5 aa, synthetic construct
  source 1..5: note = Linker
GGSGG

SEQ ID NO: 16 - protein, 21 aa, synthetic construct
  source 1..21: note = CD8 alpha signal peptide
MALPVTALLLPLALLLHAARP

SEQ ID NO: 17 - protein, 47 aa, synthetic construct
  source 1..47: note = Hinge region
KPTTTPAPRPPTPAPTIASQPLSLRPEACRPAAGGAVHTRGLDFACD

SEQ ID NO: 18 - protein, 24 aa, synthetic construct
  source 1..24: note = Transmembrane region
IYIWAPLAGTCGVLLLSLVITLYC

SEQ ID NO: 19 - protein, 41 aa, synthetic construct
  source 1..41: note = CD28 cytoplasmic domain
RSKRSRLLHSDYMNMTPRRPGPTRKHYQPYAPPRDFAAYRS

SEQ ID NO: 20 - protein, 42 aa, synthetic construct
  source 1..42: note = CD28delta cytoplasmic domain
RSKRSRLLHSDYMNMTPRRPGPTRKHYQAYAAARDFAAYRSL

SEQ ID NO: 21 - protein, 113 aa, synthetic construct
  source 1..113: note = CD3 zeta cytoplasmic domain
LRVKFSRSADAPAYQQGQNQLYNELNLGRREEYDVLDKRRGRDPEMGGKPRRKNPQEGLYNELQKDKMAEAYSEIGMKGERRRGKGHDGLYQGLSTATKDTYDALHMQALPPR

SEQ ID NO: 22 - protein, 488 aa, synthetic construct
  source 1..488: note = CAR3
MALPVTALLLPLALLLHAARPDIQMTQSPSSLSASVGDRVTITCRASQDISKYLNWYQQKPGKAPKLLIYHTSRLHSGVPSRFSGSGSGTDFTLTISSLQPEDFATYYCQQGNTLPYTFGGGTKLEIKGGGGSGGGGSGGGGSQVQLQESGPGLVKPSETLSLTCTVSGVSLPDYGVSWIRQPPGKGLEWIGVIWGSETTYYNPSLKSRVTISVDTSKNQVSLKLSSVTAADTAVYYCAKHYYYGGSYAMDYWGQGTTVTVSSKPTTTPAPRPPTPAPTIASQPLSLRPEACRPAAGGAVHTRGLDFACDIYIWAPLAGTCGVLLLSLVITLYCRSKRSRLLHSDYMNMTPRRPGPTRKHYQAYAAARDFAAYRSLRVKFSRSADAPAYQQGQNQLYNELNLGRREEYDVLDKRRGRDPEMGGKPRRKNPQEGLYNELQKDKMAEAYSEIGMKGERRRGKGHDGLYQGLSTATKDTYDALHMQALPPR

SEQ ID NO: 23 - protein, 488 aa, synthetic construct
  source 1..488: note = CAR24
MALPVTALLLPLALLLHAARPDIQMTQSPSSLSASVGDRVTITCRASQDISKYLNWYQQKPGKAPKLLIYHTSRLHSGVPSRFSGSGSGTDFTLTISSLQPEDFATYYCQQGNTLPYTFGGGTKLEIKGGGGSGGGGSGGGGSQVQLQESGPGLVKPSETLSLTCTVSGVSLPDYGVSWIRQPPGKGLEWIGVIWGSETTYYNPSLKSRVTISVDTSKNQVSLKLSSVTAADTAVYYCAKHYYYGGSYAMDYWGQGTTVTVSSKPTTTPAPRPPTPAPTIASQPLSLRPEACRPAAGGAVHTRGLDFACDIYIWAPLAGTCGVLLLSLVITLYCRSKRSRLLHSDYMNMTPRRPGPTRKHYQPYAPPRDFAAYRSLRVKFSRSADAPAYQQGQNQLYNELNLGRREEYDVLDKRRGRDPEMGGKPRRKNPQEGLYNELQKDKMAEAYSEIGMKGERRRGKGHDGLYQGLSTATKDTYDALHMQALPPR

SEQ ID NO: 24 - protein, 488 aa, synthetic construct
  source 1..488: note = CAR1
MALPVTALLLPLALLLHAARPDIQMTQSPSSLSASVGDRVTISCRASQDISKYLNWYQQKPGKAPKLLIYHTSRLHSGVPSRFSGSGSGTDYTLTISSLQPEDFATYYCQQGNTLPYTFGGGTKLEIKGGGGSGGGGSGGGGSEVQLQESGPGLVKPSETLSVTCTVSGVSLPDYGVSWIRQPPGKGLEWLGVIWGSETTYYNSALKSRLTIIKDNSKSQVFLKMSSLTAADTAVYYCAKHYYYGGSYAMDYWGQGTTVTVSSKPTTTPAPRPPTPAPTIASQPLSLRPEACRPAAGGAVHTRGLDFACDIYIWAPLAGTCGVLLLSLVITLYCRSKRSRLLHSDYMNMTPRRPGPTRKHYQAYAAARDFAAYRSLRVKFSRSADAPAYQQGQNQLYNELNLGRREEYDVLDKRRGRDPEMGGKPRRKNPQEGLYNELQKDKMAEAYSEIGMKGERRRGKGHDGLYQGLSTATKDTYDALHMQALPPR

SEQ ID NO: 25 - protein, 488 aa, synthetic construct
  source 1..488: note = CAR2
MALPVTALLLPLALLLHAARPDIQMTQSPSSLSASVGDRVTISCRASQDISKYLNWYQQKPGKAPKLLIYHTSRLHSGVPSRFSGSGSGTDYTLTISSLQPEDFATYYCQQGNTLPYTFGGGTKLEIKGGGGSGGGGSGGGGSQVQLQESGPGLVKPSETLSLTCTVSGVSLPDYGVSWIRQPPGKGLEWLGVIWGSETTYYNSALKSRLTISKDNSKSQVFLKMSSVTAADTAVYYCAKHYYYGGSYAMDYWGQGTTVTVSSKPTTTPAPRPPTPAPTIASQPLSLRPEACRPAAGGAVHTRGLDFACDIYIWAPLAGTCGVLLLSLVITLYCRSKRSRLLHSDYMNMTPRRPGPTRKHYQAYAAARDFAAYRSLRVKFSRSADAPAYQQGQNQLYNELNLGRREEYDVLDKRRGRDPEMGGKPRRKNPQEGLYNELQKDKMAEAYSEIGMKGERRRGKGHDGLYQGLSTATKDTYDALHMQALPPR